European Patent Application EP 4 516 932 A1, published March 5, 2025. Title: 시험관 진화 기반 핫스팟 유래 펩타이드-핵산 하이브리드 분자 제조방법. Applicant: POSTECH Research and Business Development Foundation. The sequence listing filed with the application follows.

SEQUENCE LISTING (22 sequences)

SEQ ID NO: 1 - DNA, 15 bp, synthetic construct
  source 1..15: mol_type = other DNA
ggaagagatggcgac

SEQ ID NO: 2 - DNA, 15 bp, synthetic construct
  source 1..15: mol_type = other DNA
ccatcaggatcagct

SEQ ID NO: 3 - DNA, 70 bp, synthetic construct
  source 1..70: mol_type = other DNA
ggaagagatggcgacnnnnnnnnnnnnnnnnnnnnnnnnnnnnnnnnnnnnnnnnagctgatcctgatgg

SEQ ID NO: 4 - DNA, 92 bp, synthetic construct
  source 1..92: mol_type = other DNA
aatgatacggcgaccaccgagatctacacttggtgagacactctttccctacacgacgctcttccgatctnnnnnnnggaagagatggcgac

SEQ ID NO: 5 - DNA, 87 bp, synthetic construct
  source 1..87: mol_type = other DNA
caagcagaagacggcatacgagatgttcaggtctgactggagttcagacgtgtgctcttccgatctnnnnnnccatcaggatcagct

SEQ ID NO: 6 - DNA, 65 bp, synthetic construct
  source 1..65: mol_type = other DNA
ggaagagatggcgacctccacaaccgctgatcgacgcagatcttgtgggtagctgatcctgatgg

SEQ ID NO: 7 - DNA, 60 bp, synthetic construct
  source 1..60: mol_type = other DNA
ggaagagatggcgacacgcaatcgtgggttggggatataatggtaagctgatcctgatgg

SEQ ID NO: 8 - DNA, 60 bp, synthetic construct; identical to SEQ ID NO: 7
  source 1..60: mol_type = other DNA

SEQ ID NO: 9 - DNA, 60 bp, synthetic construct
  source 1..60: mol_type = other DNA
ggaagagatggcgaccacaccaaatctgagtctaccccatgaaggagctgatcctgatgg

SEQ ID NO: 10 - DNA, 51 bp, synthetic construct
  source 1..51: mol_type = other DNA
cagcaccgaccttgtgctttgggagtgctggtccaagggcgttaatggaca

SEQ ID NO: 11 - DNA, 46 bp, synthetic construct
  source 1..46: mol_type = other DNA
cgcagcacccaagaacaaggactgcttaggattgcgataggttcgg

SEQ ID NO: 12 - DNA, 40 bp, synthetic construct
  source 1..40: mol_type = other DNA
tcgagtggcttgtttgtaatgtagggttccggtcgtgggt

SEQ ID NO: 13 - DNA, 60 bp, synthetic construct; identical to SEQ ID NO: 7
  source 1..60: mol_type = other DNA
  misc_difference 2..5: note = 2'-O-Methyl modified
  misc_difference 56..58: note = 2'-O-Methyl modified
  misc_difference 59: note = 2'-F modified

SEQ ID NO: 14 - DNA, 60 bp, synthetic construct; identical to SEQ ID NO: 7
  source 1..60: mol_type = other DNA
  misc_difference 1..4: note = Phosphorothioate modified
  misc_difference 56..59: note = Phosphorothioate modified

SEQ ID NO: 15 - protein, 7 aa, synthetic construct
LGKGDFR

SEQ ID NO: 16 - DNA, 35 bp, synthetic construct
  source 1..35: mol_type = other DNA
ctccacaaccgctgatcgacgcagatcttgtgggt

SEQ ID NO: 17 - DNA, 34 bp, synthetic construct
  source 1..34: mol_type = other DNA
ctccacaaccgctgatcgacgcagatcttgtggt

SEQ ID NO: 18 - DNA, 30 bp, synthetic construct
  source 1..30: mol_type = other DNA
acgcaatcgtgggttggggatataatggta

SEQ ID NO: 19 - DNA, 30 bp, synthetic construct
  source 1..30: mol_type = other DNA
acgcaatcgtgggttggggacataatggta

SEQ ID NO: 20 - DNA, 29 bp, synthetic construct
  source 1..29: mol_type = other DNA
acgcaatcgtgggttgggatataatggta

SEQ ID NO: 21 - DNA, 30 bp, synthetic construct
  source 1..30: mol_type = other DNA
cacaccaaatctgagtctaccccatgaagg

SEQ ID NO: 22 - DNA, 30 bp, synthetic construct
  source 1..30: mol_type = other DNA
cacaccaaatctgagtctaccctatgaagg